European Patent Specification EP 4 208 481 B1, published March 4, 2026. Title: ANTI-CEACAM5 ANTIBODIES AND CONJUGATES AND USES THEREOF. Applicant: Merck Patent GmbH. The sequence listing filed with the application follows.

SEQUENCE LISTING (30 sequences)

SEQ ID NO: 1 - protein, 702 aa, Homo sapiens
  Human CEACAM5 protein sequence according to GenBank accession number AAA51967.1
MESPSAPPHRWCIPWQRLLLTASLLTFWNPPTTAKLTIESTPFNVAEGKEVLLLVHNLPQHLFGYSWYKGERVDGNRQIIGYVIGTQQATPGPAYSGREIIYPNASLLIQNIIQNDTGFYTLHVIKSDLVNEEATGQFRVYPELPKPSISSNNSKPVEDKDAVAFTCEPETQDATYLWWVNNQSLPVSPRLQLSNGNRTLTLFNVTRNDTASYKCETQNPVSARRSDSVILNVLYGPDAPTISPLNTSYRSGENLNLSCHAASNPPAQYSWFVNGTFQQSTQELFIPNITVNNSGSYTCQAHNSDTGLNRTTVTTITVYAEPPKPFITSNNSNPVEDEDAVALTCEPEIQNTTYLWWVNNQSLPVSPRLQLSNDNRTLTLLSVTRNDVGPYECGIQNELSVDHSDPVILNVLYGPDDPTISPSYTYYRPGVNLSLSCHAASNPPAQYSWLIDGNIQQHTQELFISNITEKNSGLYTCQANNSASGHSRTTVKTITVSAELPKPSISSNNSKPVEDKDAVAFTCEPEAQNTTYLWWVNGQSLPVSPRLQLSNGNRTLTLFNVTRNDARAYVCGIQNSVSANRSDPVTLDVLYGPDTPIISPPDSSYLSGANLNLSCHSASNPSPQYSWRINGIPQQHTQVLFIAKITPNNNGTYACFVSNLATGRNNSIVKSITVSASGTSPGLSAGATVGIMIGVLVGVALI

SEQ ID NO: 2 - protein, 705 aa, Macaca fascicularis
  Macaca fascicularis CEACAM5 protein sequence (NCBI Reference Sequence XP_005589491.1)
MGSPSAPLHRWCIPWQTLLLTASLLTFWNPPTTAQLTIESRPFNVAEGKEVLLLAHNVSQNLFGYIWYKGERVDASRRIGSCVIRTQQITPGPAHSGRETIDFNASLLIHNVTQSDTGSYTIQVIKEDLVNEEATGQFRVYPELPKPYISSNNSNPVEDKDAVALTCEPETQDTTYLWWVNNQSLPVSPRLELSSDNRTLTVFNIPRNDTTSYKCETQNPVSVRRSDPVTLNVLYGPDAPTISPLNTPYRAGENLNLSCHAASNPTAQYFWFVNGTFQQSTQELFIPNITVNNSGSYMCQAHNSATGLNRTTVTAITVYAELPKPYITSNNSNPIEDKDAVTLTCEPETQDTTYLWWVNNQSLSVSSRLELSNDNRTLTVFNIPRNDTTFYECETQNPVSVRRSDPVTLNVLYGPDAPTISPLNTPYRAGENLNLSCHAASNPAAQYSWFVNGTFQQSTQELFIPNITVNNSGSYMCQAHNSATGLNRTTVTAITVYVELPKPYISSNNSNPIEDKDAVTLTCEPVAENTTYLWWVNNQSLSVSPRLQLSNGNRILTLLSVTRNDTGPYECGIQNSESAKRSDPVTLNVTYGPDTPIISPPDLSYRSGANLNLSCHSDSNPSPQYSWLINGTLRQHTQVLFISKITSNNNGAYACFVSNLATGRNNSIVKNISVSSGDSAPGSSGLSARATVGIIIGMLVGVALM

SEQ ID NO: 3 - protein, 10 aa, Artificial Sequence
  CDR1-H of mAb1
DGSVSRGGYY

SEQ ID NO: 4 - protein, 7 aa, Artificial Sequence
  CDR2-H of mAb1
IYYSGST

SEQ ID NO: 5 - protein, 11 aa, Artificial Sequence
  CDR3-H of mAb1
ARGIAVAPFDY

SEQ ID NO: 6 - protein, 6 aa, Artificial Sequence
  CDR1-L of mAb1
QSVRSN

SEQ ID NO: 7 - protein, 3 aa, Artificial Sequence
  CDR2-L of mAb1
AAS

SEQ ID NO: 8 - protein, 9 aa, Artificial Sequence
  CDR3-L of mAb1
QQYTNWPFT

SEQ ID NO: 9 - protein, 119 aa, Artificial Sequence
  VH of mAb1
EVQLQESGPGLVKPSQTLSLTCTVSDGSVSRGGYYLTWIRQHPGKGLEWIGYIYYSGSTYFNPSLRSRVTMSVDTSKNQFSLKLSSVTAADTAVYYCARGIAVAPFDYWGQGTLVTVSS

SEQ ID NO: 10 - protein, 107 aa, Artificial Sequence
  VL of mAb1
EIVLTQSPATLSVSPGERATLSCRTSQSVRSNLAWYQQKPGQAPRLLIYAASTRATGIPARFSGSGSGTEFTLTISSLQSEDFAVYYCQQYTNWPFTFGPGTKVDIK

SEQ ID NO: 11 - protein, 328 aa, Artificial Sequence
  CH of mAb1
ASTKGPSVFPLAPSSKSTSGGTAALGCLVKDYFPEPVTVSWNSGALTSGVHTFPAVLQSSGLYSLSSVVTVPSSSLGTQTYICNVNHKPSNTKVDKRVEPKSCDKTHTCPPCPAPPVAGPSVFLFPPKPKDTLMISRTPEVTCVVVDVSHEDPEVKFNWYVDGVEVHNAKTKPREEQYNSTYRVVSVLTVLHQDWLNGKEYKCKVSNKALPSSIEKTISKAKGQPREPQVYTLPPSREEMTKNQVSLTCLVKGFYPSDIAVEWESNGQPENNYKTTPPVLDSDGSFFLYSKLTVDKSRWQQGNVFSCSVMHEALHNHYTQKSLSLSPG

SEQ ID NO: 12 - protein, 107 aa, Artificial Sequence [sequence omitted]

SEQ ID NO: 13 - protein, 447 aa, Artificial Sequence
  HC of mAb1
EVQLQESGPGLVKPSQTLSLTCTVSDGSVSRGGYYLTWIRQHPGKGLEWIGYIYYSGSTYFNPSLRSRVTMSVDTSKNQFSLKLSSVTAADTAVYYCARGIAVAPFDYWGQGTLVTVSSASTKGPSVFPLAPSSKSTSGGTAALGCLVKDYFPEPVTVSWNSGALTSGVHTFPAVLQSSGLYSLSSVVTVPSSSLGTQTYICNVNHKPSNTKVDKRVEPKSCDKTHTCPPCPAPPVAGPSVFLFPPKPKDTLMISRTPEVTCVVVDVSHEDPEVKFNWYVDGVEVHNAKTKPREEQYNSTYRVVSVLTVLHQDWLNGKEYKCKVSNKALPSSIEKTISKAKGQPREPQVYTLPPSREEMTKNQVSLTCLVKGFYPSDIAVEWESNGQPENNYKTTPPVLDSDGSFFLYSKLTVDKSRWQQGNVFSCSVMHEALHNHYTQKSLSLSPG

SEQ ID NO: 14 - protein, 214 aa, Artificial Sequence
  LC of mAb1
EIVLTQSPATLSVSPGERATLSCRTSQSVRSNLAWYQQKPGQAPRLLIYAASTRATGIPARFSGSGSGTEFTLTISSLQSEDFAVYYCQQYTNWPFTFGPGTKVDIKRTVAAPSVFIFPPSDEQLKSGTASVVCLLNNFYPREAKVQWKVDNALQSGNSQESVTEQDSKDSTYSLSSTLTLSKADYEKHKVYACEVTHQGLSSPVTKSFNRGEC

SEQ ID NO: 15 - DNA, 1404 bp, Artificial Sequence
  DNA sequence encoding HC of mAb1
atggagaccgacaccctgctgctgtgggtgctgctgctgtgggtgcccgggtcgaccggtgaggtgcagctgcaggagtcgggcccaggactggtgaagccttcacagaccctgtccctcacctgcactgtctctgatggctccgtcagcaggggtggttactacttgacctggatccgccagcacccagggaagggcctggagtggattgggtacatctattacagtgggagcacctacttcaacccgtccctcaggagtcgggttaccatgtcagtagacacgtctaagaaccagttctccctgaagctgagctctgtgactgccgcggacacggccgtgtattactgtgcgagagggatagcagtggctccctttgactactggggccagggaaccctggtcaccgtctcttcagctagcaccaagggccccagcgtgttccccctggcccccagcagcaagtccacaagcggaggaacagccgccctgggctgcctggtgaaggactacttccccgagcccgtgaccgtgtcctggaacagcggagccctgacctccggcgtgcacaccttccccgccgtgctgcagagcagcggcctgtacagcctgagcagcgtggtgacagtgccaagcagcagcctgggaacccagacctacatctgcaacgtgaaccacaagcccagcaacaccaaggtggacaagagagtggagcccaagagctgcgacaagacccatacctgtccaccctgcccagcccccccagtggccggaccctccgtgttcctgttcccccccaagcccaaggacaccctgatgatcagcaggacccccgaggtgacctgcgtggtggtggacgtgagccacgaggacccagaggtgaagttcaattggtatgtggacggcgtggaggtgcacaacgccaagaccaagcccagagaggaacagtacaacagcacctacagggtggtgtccgtgctgaccgtgctgcaccaggactggctgaacggcaaggaatacaagtgcaaggtctccaacaaggccctgccctccagcatcgagaaaaccatcagcaaggccaagggccagccacgggagccccaggtgtacacactgcccccatctcgggaagaaatgaccaagaaccaggtgtccctgacctgtctggtgaagggcttttaccccagcgacatcgccgtggagtgggagagcaacggccagcccgagaacaactacaagaccaccccccctgtgctggacagcgacggcagcttcttcctgtacagcaagctgaccgtggacaagtccaggtggcagcagggcaacgtgttcagctgcagcgtgatgcacgaggccctgcacaaccactacacacagaagagcctgagcctgtcccccggctga

SEQ ID NO: 16 - DNA, 708 bp, Artificial Sequence
  DNA sequence encoding LC of mAb1
atgagggccctgctggctagactgctgctgtgcgtgctggtcgtgtccgacagcaagggcgaaatcgtactcacgcagtctccagccaccctgtctgtgtctccaggggaaagagccaccctctcctgcaggaccagtcagagtgttcgcagcaacttagcctggtaccagcagaagcctggccaggctcccaggctcctcatctatgctgcatccaccagggccactggtatcccagccaggttcagtggcagtgggtctgggacagagttcactctcaccatcagcagcctgcagtctgaagattttgcagtttattactgtcagcagtatactaactggccattcactttcggccctgggaccaaagtggacatcaaacgtacggtggctgcaccatctgtcttcatcttcccgccatctgatgagcagttgaaatctggaactgcctctgttgtgtgcctgctgaataacttctatcccagagaggccaaagtacagtggaaggtggataacgccctccaatcgggtaactcccaggagagtgtcacagagcaggacagcaaggacagcacctacagcctcagcagcaccctgacgctgagcaaagcagactacgagaaacacaaagtctacgcctgcgaagtcacccatcagggcctgagctcgcccgtcacaaagagcttcaacaggggagagtgttgatag

SEQ ID NO: 17 - protein, 449 aa, Artificial Sequence
  HC of antibody hu8G4
EVQLVESGPGLVKPSQTLSLTCTVSDGSVSRGGYYLTWIRQHPGKGLEWIGYIYYSGSTYFNPSLRSRLTMSVDTSKNQFSLKLSSVTAADTAVYYCARGIAVAPFDYWGQGTLVTVSSASTKGPSVFPLAPSSKSTSGGTAALGCLVKDYFPEPVTVSWNSGALTSGVHTFPAVLQSSGLYSLSSVVTVPSSSLGTQTYICNVNHKPSNTKVDKRVEPKSCDKTHTCPPCPAPELLGGPSVFLFPPKPKDTLMISRTPEVTCVVVDVSHEDPEVKFNWYVDGVEVHNAKTKPREEQYNSTYRVVSVLTVLHQDWLNGKEYKCKVSNKALPAPIEKTISKAKGQPREPQVYTLPPSREEMTKNQVSLTCLVKGFYPSDIAVEWESNGQPENNYKTTPPVLDSDGSFFLYSKLTVDKSRWQQGNVFSCSVMHEALHNHYTQKSLSLSPGK

SEQ ID NO: 18 - protein, 214 aa, Artificial Sequence
  LC of antibody hu8G4
ETTLTQSPATLSVSPGERATLSCRTSQSVRSNLAWYQQKPGQAPRLLIYAASTRATGIPARFSGSGSGTEFTLTIGSLQSEDFAVYFCQQYTNWPFTFGPGTKVEIKRTVAAPSVFIFPPSDEQLKSGTASVVCLLNNFYPREAKVQWKVDNALQSGNSQESVTEQDSKDSTYSLSSTLTLSKADYEKHKVYACEVTHQGLSSPVTKSFNRGEC

SEQ ID NO: 19 - protein, 449 aa, Artificial Sequence
  HC of optimized antibody Variant 1
EVQLQESGPGLVKPSQTLSLTCTVSDGSVSRGGYYLTWIRQHPGKGLEWIGYIYYSGSTYFNPSLRSRLTMSVDTSKNQFSLKLSSVTAADTAVYYCARGIAVAPFDYWGQGTLVTVSSASTKGPSVFPLAPSSKSTSGGTAALGCLVKDYFPEPVTVSWNSGALTSGVHTFPAVLQSSGLYSLSSVVTVPSSSLGTQTYICNVNHKPSNTKVDKRVEPKSCDKTHTCPPCPAPELLGGPSVFLFPPKPKDTLMISRTPEVTCVVVDVSHEDPEVKFNWYVDGVEVHNAKTKPREEQYNSTYRVVSVLTVLHQDWLNGKEYKCKVSNKALPAPIEKTISKAKGQPREPQVYTLPPSREEMTKNQVSLTCLVKGFYPSDIAVEWESNGQPENNYKTTPPVLDSDGSFFLYSKLTVDKSRWQQGNVFSCSVMHEALHNHYTQKSLSLSPGK

SEQ ID NO: 20 - protein, 214 aa, Artificial Sequence; identical to SEQ ID NO: 18
  LC of optimized antibody Variant 1

SEQ ID NO: 21 - protein, 214 aa, Artificial Sequence
  LC of optimized antibody Variant 2
EIVLTQSPATLSVSPGERATLSCRTSQSVRSNLAWYQQKPGQAPRLLIYAASTRATGIPARFSGSGSGTEFTLTISSLQSEDFAVYFCQQYTNWPFTFGPGTKVDIKRTVAAPSVFIFPPSDEQLKSGTASVVCLLNNFYPREAKVQWKVDNALQSGNSQESVTEQDSKDSTYSLSSTLTLSKADYEKHKVYACEVTHQGLSSPVTKSFNRGEC

SEQ ID NO: 22 - protein, 214 aa, Artificial Sequence
  LC of optimized antibody Variant 4
EIVMTQSPATLSVSPGERATLSCRTSQSVRSNLAWYQQKPGQAPRLLIYAASTRATGIPARFSGSGSGTEFTLTISSLQSEDFAVYFCQQYTNWPFTFGPGTKVDIKRTVAAPSVFIFPPSDEQLKSGTASVVCLLNNFYPREAKVQWKVDNALQSGNSQESVTEQDSKDSTYSLSSTLTLSKADYEKHKVYACEVTHQGLSSPVTKSFNRGEC

SEQ ID NO: 23 - protein, 214 aa, Artificial Sequence
  LC of optimized antibody Variant 5
EIVMTQSPATLSVSPGERATLSCRTSQSVRSNLAWYQQKPGQAPRLLIYAASTRATGIPARFSGSGSGTEFTLTISSLQSEDFAVYYCQQYTNWPFTFGPGTKVDIKRTVAAPSVFIFPPSDEQLKSGTASVVCLLNNFYPREAKVQWKVDNALQSGNSQESVTEQDSKDSTYSLSSTLTLSKADYEKHKVYACEVTHQGLSSPVTKSFNRGEC

SEQ ID NO: 24 - protein, 449 aa, Artificial Sequence
  HC of optimized antibody Variant 6
EVQLQESGPGLVKPSQTLSLTCTVSDGSVSRGGYYLTWIRQHPGKGLEWIGYIYYSGSTYFNPSLRSRVTMSVDTSKNQFSLKLSSVTAADTAVYYCARGIAVAPFDYWGQGTLVTVSSASTKGPSVFPLAPSSKSTSGGTAALGCLVKDYFPEPVTVSWNSGALTSGVHTFPAVLQSSGLYSLSSVVTVPSSSLGTQTYICNVNHKPSNTKVDKRVEPKSCDKTHTCPPCPAPELLGGPSVFLFPPKPKDTLMISRTPEVTCVVVDVSHEDPEVKFNWYVDGVEVHNAKTKPREEQYNSTYRVVSVLTVLHQDWLNGKEYKCKVSNKALPAPIEKTISKAKGQPREPQVYTLPPSREEMTKNQVSLTCLVKGFYPSDIAVEWESNGQPENNYKTTPPVLDSDGSFFLYSKLTVDKSRWQQGNVFSCSVMHEALHNHYTQKSLSLSPGK

SEQ ID NO: 25 - protein, 450 aa, Artificial Sequence
  HC of huMab2-3 (allotype)
EVQLQESGPGLVKPGGSLSLSCAASGFVFSSYDMSWVRQTPERGLEWVAYISSGGGITYAPSTVKGRFTVSRDNAKNTLYLQMNSLTSEDTAVYYCAAHYFGSSGPFAYWGQGTLVTVSSASTKGPSVFPLAPSSKSTSGGTAALGCLVKDYFPEPVTVSWNSGALTSGVHTFPAVLQSSGLYSLSSVVTVPSSSLGTQTYICNVNHKPSNTKVDKRVEPKSCDKTHTCPPCPAPELLGGPSVFLFPPKPKDTLMISRTPEVTCVVVDVSHEDPEVKFNWYVDGVEVHNAKTKPREEQYNSTYRVVSVLTVLHQDWLNGKEYKCKVSNKALPAPIEKTISKAKGQPREPQVYTLPPSREEMTKNQVSLTCLVKGFYPSDIAVEWESNGQPENNYKTTPPVLDSDGSFFLYSKLTVDKSRWQQGNVFSCSVMHEALHNHYTQKSLSLSPGK

SEQ ID NO: 26 - protein, 214 aa, Artificial Sequence
  LC of huMab2-3
DIQMTQSPASLSASVGDRVTITCRASENIFSYLAWYQQKPGKSPKLLVYNTRTLAEGVPSRFSGSGSGTDFSLTISSLQPEDFATYYCQHHYGTPFTFGSGTKLEIKRTVAAPSVFIFPPSDEQLKSGTASVVCLLNNFYPREAKVQWKVDNALQSGNSQESVTEQDSKDSTYSLSSTLTLSKADYEKHKVYACEVTHQGLSSPVTKSFNRGEC

SEQ ID NO: 27 - protein, 449 aa, Artificial Sequence
  HC of hmn-14
EVQLVESGGGVVQPGRSLRLSCSASGFDFTTYWMSWVRQAPGKGLEWIGEIHPDSSTINYAPSLKDRFTISRDNAKNTLFLQMDSLRPEDTGVYFCASLYFGFPWFAYWGQGTPVTVSSASTKGPSVFPLAPSSKSTSGGTAALGCLVKDYFPEPVTVSWNSGALTSGVHTFPAVLQSSGLYSLSSVVTVPSSSLGTQTYICNVNHKPSNTKVDKRVEPKSCDKTHTCPPCPAPELLGGPSVFLFPPKPKDTLMISRTPEVTCVVVDVSHEDPEVKFNWYVDGVEVHNAKTKPREEQYNSTYRVVSVLTVLHQDWLNGKEYKCKVSNKALPAPIEKTISKAKGQPREPQVYTLPPSREEMTKNQVSLTCLVKGFYPSDIAVEWESNGQPENNYKTTPPVLDSDGSFFLYSKLTVDKSRWQQGNVFSCSVMHEALHNHYTQKSLSLSPGK

SEQ ID NO: 28 - protein, 213 aa, Artificial Sequence
  LC of hmn-14
DIQLTQSPSSLSASVGDRVTITCKASQDVGTSVAWYQQKPGKAPKLLIYWTSTRHTGVPSRFSGSGSGTDFTFTISSLQPEDIATYYCQQYSLYRSFGQGTKVEIKRTVAAPSVFIFPPSDEQLKSGTASVVCLLNNFYPREAKVQWKVDNALQSGNSQESVTEQDSKDSTYSLSSTLTLSKADYEKHKVYACEVTHQGLSSPVTKSFNRGEC

SEQ ID NO: 29 - protein, 441 aa, Artificial Sequence
  HC of rb8G4
EVQLQESGPGLVKPSQTLSLTCTVSDGSVSRGGYYLTWIRQHPGKGLEWIGYIYYSGSTYFNPSLRSRVTMSVDTSKNQFSLKLSSVTAADTAVYYCARGIAVAPFDYWGQGTLVTVSSQPKAPSVFPLAPCCGDTPSSTVTLGCLVKGYLPEPVTVTWNSGTLTNGVRTFPSVRQSSGLYSLSSVVSVTSSSQPVTCNVAHPATNTKVDKTVAPSTCSKPTCPPPELLGGPSVFIFPPKPKDTLMISRTPEVTCVVVDVSEDDPEVQFTWYINNEQVRTARPPLREQQFNSTIRVVSTLPIAHEDWLRGKEFKCKVHNKALPAPIEKTISKARGQPLEPKVYTMGPPREELSSRSVSLTCMINGFYPSDISVEWEKNGKAEDNYKTTPAVLDSDGSYFLYSKLSVPTSEWQRGDVFTCSVMHEALHNHYTQKSISRSPGK

SEQ ID NO: 30 - protein, 213 aa, Artificial Sequence
  LC of rb8G4
EIVLTQSPATLSVSPGERATLSCRTSQSVRSNLAWYQQKPGQAPRLLIYAASTRATGIPARFSGSGSGTEFTLTISSLQSEDFAVYYCQQYTNWPFTFGPGTKVDIKRDPVAPSVLLFPPSKEELTTGTATIVCVANKFYPSDITVTWKVDGTTQQSGIENSKTPQSPEDNTYSLSSTLSLTSAQYNSHSVYTCEVVQGSASPIVQSFNRGDC